European Patent Application EP 4 446 435 A1, published October 16, 2024. Title: Method of detecting mutants in a sequence of interest, method of inhibiting nucleic acid amplification, kit for carrying out the methods, and agent for enhancing amplification inhibitory effect. Applicant: 日東紡績株式会社. The sequence listing filed with the application follows.

SEQUENCE LISTING (15 sequences)

SEQ ID NO: 1 - DNA, 24 bp, synthetic construct
  misc_feature 1..24: note = Forward primer
  source 1..24: mol_type = other DNA
gcctgctgaaaatgactgaatata

SEQ ID NO: 2 - DNA, 23 bp, synthetic construct
  misc_feature 1..23: note = Reverse primer
  source 1..23: mol_type = other DNA
caagatttacctctattgttgga

SEQ ID NO: 3 - DNA, 132 bp, HCC70 strain genome
  misc_feature 1..132: note = Template DNA
  source 1..132: mol_type = genomic DNA
gcctgctgaaaatgactgaatataaacttgtggtagttggagctggtggcgtaggcaagagtgccttgacgatacagctaattcagaatcattttgtggacgaatatgatccaacaatagaggtaaatcttg

SEQ ID NO: 4 - DNA, 300 bp, HCC70 strain genome
  source 1..300: mol_type = genomic DNA
tgagtttgtattaaaaggtactggtggagtatttgatagtgtattaaccttatgtgtgacatgttctaatatagtcacattttcattatttttattataaggcctgctgaaaatgactgaatataaacttgtggtagttggagctggtggcgtaggcaagagtgccttgacgatacagctaattcagaatcattttgtggacgaatatgatccaacaatagaggtaaatcttgttttaatatgcatattactggtgcaggaccattctttgatacacgataaaggtttctctgaccattt

SEQ ID NO: 5 - DNA, 25 bp, synthetic construct
  misc_feature 1..25: note = Forward primer
  source 1..25: mol_type = other DNA
ctgaatataaacttgtggtagttgg

SEQ ID NO: 6 - DNA, 20 bp, synthetic construct
  misc_feature 1..20: note = Reverse primer
  source 1..20: mol_type = other DNA
gtcctgcaccagtaatatgc

SEQ ID NO: 7 - DNA, 11 bp, synthetic construct
  misc_feature 1..2: note = 2',4'-BNANC(N-H)-cytosine
  misc_feature 3: note = 2',4'-BNANC(N-H)-thymine
  misc_feature 5: note = 2',4'-BNANC(N-H)-cytosine
  misc_feature 7..8: note = 2',4'-BNANC(N-H)-cytosine
  misc_feature 10..11: note = 2',4'-BNANC(N-H)-cytosine
  source 1..11: mol_type = other DNA
cctacgccacc

SEQ ID NO: 8 - DNA, 146 bp, HCC70 strain genome
  misc_feature 1..146: note = Template DNA
  source 1..146: mol_type = genomic DNA
ctgaatataaacttgtggtagttggagctggtggcgtaggcaagagtgccttgacgatacagctaattcagaatcattttgtggacgaatatgatccaacaatagaggtaaatcttgttttaatatgcatattactggtgcaggac

SEQ ID NO: 9 - DNA, 300 bp, HCC70 strain genome; identical to SEQ ID NO: 4
  source 1..300: mol_type = genomic DNA

SEQ ID NO: 10 - DNA, 146 bp, MDA-MB-231 strain genome
  misc_feature 1..146: note = Template DNA
  source 1..146: mol_type = genomic DNA
ctgaatataaacttgtggtagttggagctggtgacgtaggcaagagtgccttgacgatacagctaattcagaatcattttgtggacgaatatgatccaacaatagaggtaaatcttgttttaatatgcatattactggtgcaggac

SEQ ID NO: 11 - DNA, 300 bp, MDA-MB-231 strain genome
  source 1..300: mol_type = genomic DNA
tgagtttgtattaaaaggtactggtggagtatttgatagtgtattaaccttatgtgtgacatgttctaatatagtcacattttcattatttttattataaggcctgctgaaaatgactgaatataaacttgtggtagttggagctggtgacgtaggcaagagtgccttgacgatacagctaattcagaatcattttgtggacgaatatgatccaacaatagaggtaaatcttgttttaatatgcatattactggtgcaggaccattctttgatacacgataaaggtttctctgaccattt

SEQ ID NO: 12 - DNA, 300 bp, HCC70 strain genome
  source 1..300: mol_type = genomic DNA
atagaaattagatctcttacctaaactcttcataatgcttgctctgataggaaaatgagatctactgttttcctttacttactacacctcagatatatttcttcatgaagacctcacagtaaaaataggtgattttggtctagctacagtgaaatctcgatggagtgggtcccatcagtttgaacagttgtctggatccattttgtggatggtaagaattgaggctatttttccactgattaaatttttggccctgagatgctgctgagttactagaaagtcattgaaggtctcaactat

SEQ ID NO: 13 - DNA, 300 bp, DU4475 strain genome
  source 1..300: mol_type = genomic DNA
atagaaattagatctcttacctaaactcttcataatgcttgctctgataggaaaatgagatctactgttttcctttacttactacacctcagatatatttcttcatgaagacctcacagtaaaaataggtgattttggtctagctacagagaaatctcgatggagtgggtcccatcagtttgaacagttgtctggatccattttgtggatggtaagaattgaggctatttttccactgattaaatttttggccctgagatgctgctgagttactagaaagtcattgaaggtctcaactat

SEQ ID NO: 14 - DNA, 212 bp, synthetic construct
  misc_feature 1..212: note = KRAS WT plasmid
  source 1..212: mol_type = other DNA
cattatttttattataaggcctgctgaaaatgactgaatataaacttgtggtagttggagctggtggcgtaggcaagagtgccttgacgatacagctaattcagaatcattttgtggacgaatatgatccaacaatagaggtaaatcttgttttaatatgcatattactggtgcaggaccattctttgatacacgataaaggtttcaagctt

SEQ ID NO: 15 - DNA, 212 bp, synthetic construct
  misc_feature 1..212: note = KRAS Mutant plasmid
  source 1..212: mol_type = other DNA
cattatttttattataaggcctgctgaaaatgactgaatataaacttgtggtagttggagctggtgacgtaggcaagagtgccttgacgatacagctaattcagaatcattttgtggacgaatatgatccaacaatagaggtaaatcttgttttaatatgcatattactggtgcaggaccattctttgatacacgataaaggtttcaagctt